European Patent Specification EP 3 450 552 B1, published September 2, 2026. Title: IMPROVED ENZYME VARIANTS. Applicant: DSM IP ASSETS B.V. The sequence listing filed with the application follows.

SEQUENCE LISTING (2 sequences)

SEQ ID NO: 1 - DNA, 1119 bp, Bos taurus
ctcgagaaaagagctgaaatcaccagaattccattgtacaagggtaagtctttgagaaaggctttgaaggaacacggtctattggaagatttcttacaaaagcaacagtacggtatttcttccaagtactccggtttcggtgaagttgcctccgtcccattgaccaactatctggactctcaatatttcggtaagatctacttgggtactccacctcaagagttcaccgtccttttcgacactggttcttctgatttctgggttccatccatctactgtaagtccaatgcttgtaagaaccatcaaagatttgacccaagaaagtcttccactttccaaaacttgggtaagccattatccattcactatggtactggttccatgcaaggtatcttgggttacgacactgttactgtttccaacattgttgacattcaacaaaccgtcggtttgtccactcaagagcctggcgatgttttcacctacgctgaatttgatggtattttgggtatggcttacccatctttggcttctgaatactccatccctgtctttgacaacatgatgaaccgtcacttggttgctcaagatttattctccgtttacatggacagaaacggtcaagaatccatgttgactttaggtgccattgatccatcttactacactggttctctacactgggttccagttaccgtccaacaatactggcaattcaccgttgactccgtcaccatctccggtgttgttgttgcttgtgaaggtggttgccaagctatcttggacaccggtacttccaagttggtcggtccatcttctgatatcttgaacattcaacaagccattggtgccactcaaaaccagtacggtgaattcgatattgactgtgacaacttgtcttacatgccaactgttgtctttgaaatcaatggtaagatgtacccattaaccccatctgcttacacttctcaagaccaaggtttctgtacttctggtttccaatctgaaaaccattctcaaaaatggatcttgggtgatgtcttcatcagagagtactactccgtctttgaccgtgccaacaacttggttggtttggccaaggccatctaagttaattaa

SEQ ID NO: 2 - protein, 323 aa, Bos taurus
GEVASVPLTNYLDSQYFGKIYLGTPPQEFTVLFDTGSSDFWVPSIYCKSNACKNHQRFDPRKSSTFQNLGKPLSIHYGTGSMQGILGYDTVTVSNIVDIQQTVGLSTQEPGDVFTYAEFDGILGMAYPSLASEYSIPVFDNMMNRHLVAQDLFSVYMDRNGQESMLTLGAIDPSYYTGSLHWVPVTVQQYWQFTVDSVTISGVVVACEGGCQAILDTGTSKLVGPSSDILNIQQAIGATQNQYGEFDIDCDNLSYMPTVVFEINGKMYPLTPSAYTSQDQGFCTSGFQSENHSQKWILGDVFIREYYSVFDRANNLVGLAKAI